European Patent Application EP 4 424 708 A1, published September 4, 2024. Title: Antibodies derived from cancer survivors and uses thereof. Applicant: THE ASAN FOUNDATION. Application KR. The sequence listing filed with the application follows.

SEQUENCE LISTING (20 sequences)

SEQ ID NO: 1 - protein, 10 aa, synthetic construct
  REGION 1..10: note = S3-5 antibody heavy chain CDR1
GGTFSSYAIS

SEQ ID NO: 2 - protein, 17 aa, synthetic construct
  REGION 1..17: note = S3-5 antibody heavy chain CDR2
GIIPIFGTANYAQKFQG

SEQ ID NO: 3 - protein, 15 aa, synthetic construct
  REGION 1..15: note = S3-5 antibody heavy chain CDR3
EGYYDSSGPAEYFQH

SEQ ID NO: 4 - protein, 124 aa, synthetic construct
  REGION 1..124: note = S3-5 antibody heavy chain region
EVQLVQSGAEVKKPGSSVKVSCKASGGTFSSYAISWVRQAPGQGLEWMGGIIPIFGTANYAQKFQGRVTITADESTSTAYMELSSLRSEDTAVYYCAREGYYDSSGPAEYFQHWGQGTLVTVSS

SEQ ID NO: 5 - protein, 11 aa, synthetic construct
  REGION 1..11: note = S3-5 antibody light chain CDR1
AGTNIGSKSVH

SEQ ID NO: 6 - protein, 7 aa, synthetic construct
  REGION 1..7: note = S3-5 antibody light chain CDR2
NDNDRPS

SEQ ID NO: 7 - protein, 11 aa, synthetic construct
  REGION 1..11: note = S3-5 antibody light chain CDR3
QVWVSGSGEYV

SEQ ID NO: 8 - protein, 108 aa, synthetic construct
  REGION 1..108: note = S3-5 antibody light chain region
QAVLTQPPSVSVAPGKTADIACAGTNIGSKSVHWYQQKPGQAPLLVIYNDNDRPSGIPERFSGSNPGNTATLTISSVEAGDEADYYCQVWVSGSGEYVFGTGTKLTVL

SEQ ID NO: 9 - protein, 480 aa, synthetic construct
  REGION 1..480: note = S3-5 antibody full length
MAEVQLVQSGAEVKKPGSSVKVSCKASGGTFSSYAISWVRQAPGQGLEWMGGIIPIFGTANYAQKFQGRVTITADESTSTAYMELSSLRSEDTAVYYCAREGYYDSSGPAEYFQHWGQGTLVTVSSGGGGSGGGGSGGGGSQAVLTQPPSVSLAPGKTADIACAGTNIGSKSVHWYQQKPGQAPLLVIYNDNDRPSRIPERFSGSNPGNTATLTISSVEAGDEADYYCQVWVSGSGEYVFGTGTKLTVLPKSCDKTHTCPPCPAPELLGGPSVFLFPPKPKDTLMISRTPEVTCVVVDVSHEDPEVKFNWYVDGVEVHNAKTKPREEQYNSTYRVVSVLTVLHQDWLNGKEYKCKVSNKALPAPIEKTISKAKGQPREPQVYTLPPSRDELTKNQVSLTCLVKGFYPSDIAVEWESNGQPENNYKTTPPVLDSDGSFFLYSKLTVDKSRWQQGNVFSCSVMHEALHNHYTQKSLSLSPGK

SEQ ID NO: 10 - protein, 9 aa, synthetic construct
  REGION 1..9: note = S4-2 antibody heavy chain CDR1
FTFSSYDMH

SEQ ID NO: 11 - protein, 16 aa, synthetic construct
  REGION 1..16: note = S4-2 antibody heavy chain CDR2
AIGTAGDTYYPGSVKG

SEQ ID NO: 12 - protein, 8 aa, synthetic construct
  REGION 1..8: note = S4-2 antibody heavy chain CDR3
SALSAFDI

SEQ ID NO: 13 - protein, 116 aa, synthetic construct
  REGION 1..116: note = S4-2 antibody heavy chain region
QVQLVQSGGGLVQPGGSLRLSCAASGFTFSSYDMHWVRQATGKGLEWVSAIGTAGDTYYPGSVKGRFTISRDNAKNSLYLQMNSLRAEDTAVYYCARSALSAFDIWGQGTMVTVSS

SEQ ID NO: 14 - protein, 11 aa, synthetic construct
  REGION 1..11: note = S4-2 antibody light chain CDR1
RASQSISSYLN

SEQ ID NO: 15 - protein, 7 aa, synthetic construct
  REGION 1..7: note = S4-2 antibody light chain CDR2
AASTLQS

SEQ ID NO: 16 - protein, 9 aa, synthetic construct
  REGION 1..9: note = S4-2 antibody light chain CDR3
QQSYSTPRT

SEQ ID NO: 17 - protein, 107 aa, synthetic construct
  REGION 1..107: note = S4-2 antibody light chain region
DIVMTQTPSSLSVSVGDRVTITCRASQSISSYLNWYQQKPGKAPKLLIYAASTLQSGVPSRFSGSGSGTDFTLTISSLQPEDFATYYCQQSYSTPRTFGQGTKVEIK

SEQ ID NO: 18 - protein, 471 aa, synthetic construct
  REGION 1..471: note = S4-2 antibody full length
MAQVQLVQSGGGLVQPGGSLRLSCAASGFTFSSYDMHWVRQATGKGLEWVSAIGTAGDTYYPGSVKGRFTISRDNAKNSLYLQMNSLRAEDTAVYYCARSALSAFDIWGQGTMVTVSSGGGGSGGGGSGGGGSDIVMTQTPSSLSVSVGDRVTITCRASQSISSYLNWYQQKPGKAPKLLIYAASTLQSGVPSRFSGSGSGTDFTLTISSLQPEDFATYYCQQSYSTPRTFGQGTKVEIKPKSCDKTHTCPPCPAPELLGGPSVFLFPPKPKDTLMISRTPEVTCVVVDVSHEDPEVKFNWYVDGVEVHNAKTKPREEQYNSTYRVVSVLTVLHQDWLNGKEYKCKVSNKALPAPIEKTISKAKGQPREPQVYTLPPSRDELTKNQVSLTCLVKGFYPSDIAVEWESNGQPENNYKTTPPVLDSDGSFFLYSKLTVDKSRWQQGNVFSCSVMHEALHNHYTQKSLSLSPGK

SEQ ID NO: 19 - DNA, 1440 bp, synthetic construct
  misc_feature 1..1440: note = Polynucleotides encoding S3-5 antibody
  source 1..1440: mol_type = other DNA
atggccgaggtgcagctggtgcagtctggggctgaggtgaagaagcctgggtcctcggtgaaggtctcctgcaaggcttctggaggcaccttcagcagctatgctatcagctgggtgcgacaggcccctggacaagggcttgagtggatgggagggatcatccctatctttggtacagcaaactacgcacagaagttccagggcagagtcacgattaccgcggacgaatccacgagcacagcctacatggagctgagcagcctgagatctgaggacacggccgtgtattactgtgcgagagagggttactatgatagtagtggacccgctgaatacttccagcactggggccagggcaccctggtcaccgtctcctcaggtggaggaggttcaggtggaggtggatctggcggcggcggctcgcaggctgtgctgactcagccaccctcagtgtcactggccccaggaaagacggccgacattgcctgtgcgggaaccaacattggaagtaaaagtgtgcattggtaccaacagaagccaggccaggcccctctactggtcatctataatgataatgaccggccctcaaggattcctgagcgattctctggctccaaccctgggaacacggccaccctgaccatcagcagcgtcgaggccggggatgaggccgactattactgtcaggtgtgggttagtggcagtggtgaatacgtcttcggaactgggaccaagctcaccgtcctacccaaatcttgtgacaaaactcacacatgcccaccgtgcccagcacctgaactcctggggggaccgtcagtcttcctcttccccccaaaacccaaggacaccctcatgatctcccggacccctgaggtcacatgcgtggtggtggacgtgagccacgaagaccctgaggtcaagttcaactggtacgtggacggcgtggaggtgcataatgccaagacaaagccgcgggaggagcagtacaacagcacgtaccgtgtggtcagcgtcctcaccgtcctgcaccaggactggctgaatggcaaggagtacaagtgcaaggtctccaacaaagccctcccagcccccatcgagaaaaccatctccaaagccaaagggcagccccgagaaccacaggtgtacaccctgcccccatcccgggatgagctgaccaagaaccaggtcagcctgacctgcctggtcaaaggcttctatcccagcgacatcgccgtggagtgggagagcaatgggcagccggagaacaactacaagaccacgcctcccgtgctggactccgacggctccttcttcctctacagcaagctcaccgtggacaagagcaggtggcagcaggggaacgtcttctcatgctccgtgatgcatgaggctctgcacaaccactacacgcagaagagcctctccctgtccccgggtaaa

SEQ ID NO: 20 - DNA, 1413 bp, synthetic construct
  misc_feature 1..1413: note = Polynucleotides encoding S4-2 antibody
  source 1..1413: mol_type = other DNA
atggcccaagtccagctggtgcagtctgggggaggcttggtacagcctggggggtccctgagactctcctgtgcagcctctggattcaccttcagtagctacgacatgcactgggtccgccaagctacaggaaaaggtctggagtgggtctcagctattggtactgctggtgacacatactatccaggctccgtgaagggccgattcaccatctccagagacaacgccaagaactcactgtatctgcaaatgaacagcctgagagccgaggacacggctgtgtattactgtgcgagatccgccctttcggcttttgatatctggggccaagggacaatggtcaccgtctcctcaggtggaggaggttcaggtggaggtggatctggcggcggcggctcggacatcgtgatgactcagactccatcctccctgtctgtatctgtaggagacagagtcaccatcacttgccgggcaagtcagagcattagcagctatttaaattggtatcagcagaaaccagggaaagcccctaagctcctgatctatgctgcatccactttgcaaagtggggtcccatcaaggttcagcggcagtggatctgggacagatttcactctcaccatcagcagcctgcagcctgaagattttgcaacttactactgtcaacagagttacagtacccctcggacgttcggccaagggaccaaggtggagatcaaacccaaatcttgtgacaaaactcacacatgcccaccgtgcccagcacctgaactcctggggggaccgtcagtcttcctcttccccccaaaacccaaggacaccctcatgatctcccggacccctgaggtcacatgcgtggtggtggacgtgagccacgaagaccctgaggtcaagttcaactggtacgtggacggcgtggaggtgcataatgccaagacaaagccgcgggaggagcagtacaacagcacgtaccgtgtggtcagcgtcctcaccgtcctgcaccaggactggctgaatggcaaggagtacaagtgcaaggtctccaacaaagccctcccagcccccatcgagaaaaccatctccaaagccaaagggcagccccgagaaccacaggtgtacaccctgcccccatcccgggatgagctgaccaagaaccaggtcagcctgacctgcctggtcaaaggcttctatcccagcgacatcgccgtggagtgggagagcaatgggcagccggagaacaactacaagaccacgcctcccgtgctggactccgacggctccttcttcctctacagcaagctcaccgtggacaagagcaggtggcagcaggggaacgtcttctcatgctccgtgatgcatgaggctctgcacaaccactacacgcagaagagcctctccctgtccccgggtaaa